European Patent Specification EP 3 043 836 B1, published May 10, 2023. Title: Encapsulated Cell Therapy Cartridge. Applicant: Neurotech USA, Inc. Application EP14776945.9. The sequence listing filed with the application follows.

SEQUENCE LISTING (32 sequences)

SEQ ID NO: 1 - DNA, 1401 bp, Artificial Sequence
  834 molecule nucleic acid sequence
atggtcagctactgggacaccggggtcctgctgtgcgcgctgctcagctgtctgcttctcacaggatctagttcaggttcgcgaagtgatacaggtagacctttcgtagagatgtacagtgaaatccccgaaattatacacatgactgaaggaagggagctcgtcattccctgccgggttacgtcacctaacatcactgttactttaaaaaagtttccacttgacactttgatccctgatggaaaacgcataatctgggacagtagaaagggcttcatcatatcaaatgcaacgtacaaagaaatagggcttctgacctgtgaagcaacagtcaatgggcatttgtataagacaaactatctcacacatcgacaaaccaatacaatcatcgatgtggttctgagtccgtctcatggaattgaactatctgttggagaaaagcttgtcttaaattgtacagcaagaactgaactaaatgtggggattgacttcaactgggaatacccttcttcgaagcatcagcataagaaacttgtaaaccgagacctaaaaacccagtctgggagtgagatgaagaaatttttgagcaccttaactatagatggtgtaacccggagtgaccaaggattgtacacctgtgcagcatccagtgggctgatgaccaagaagaacagcacatttgtcagggtccatgaaaaagaattcgagcccaaatcttgtgacaaaactcacacatgcccaccgtgcccagcacctgaactcctggggggaccgtcagtcttcctcttccccccaaaacccaaggacaccctcatgatctcccggacccctgaggtcacatgcgtggtggtggacgtgagccacgaagaccctgaggtcaagttcaactggtacgtggacggcgtggaggtgcataatgccaagacaaagccgcgggaggagcagtacaacagcacgtaccgtgtggtcagcgtcctcaccgtcctgcaccaggactggctgaatggcaaggagtacaagtgcaaggtctccaacaaagccctcccagcccccatcgagaaaaccatctccaaagccaaagggcagccccgagaaccacaggtgtacaccctgcccccatcccgggatgagctgaccaagaaccaggtcagcctgacctgcctggtcaaaggcttctatcccagcgacatcgccgtggagtgggagagcaatgggcagccggagaacaactacaagaccacgcctcccgtgctggactccgacggctccttcttcctctacagcaagctcaccgtggacaagagcaggtggcagcaggggaacgtcttctcatgctccgtgatgcatgaggctctgcacaaccactacacgcagaagagcctctccctgtctccgggtaaa

SEQ ID NO: 2 - protein, 467 aa, Artificial Sequence
  834 molecule amino acid sequence
MVSYWDTGVLLCALLSCLLLTGSSSGSRSDTGRPFVEMYSEIPEIIHMTEGRELVIPCRVTSPNITVTLKKFPLDTLIPDGKRIIWDSRKGFIISNATYKEIGLLTCEATVNGHLYKTNYLTHRQTNTIIDVVLSPSHGIELSVGEKLVLNCTARTELNVGIDFNWEYPSSKHQHKKLVNRDLKTQSGSEMKKFLSTLTIDGVTRSDQGLYTCAASSGLMTKKNSTFVRVHEKEFEPKSCDKTHTCPPCPAPELLGGPSVFLFPPKPKDTLMISRTPEVTCVVVDVSHEDPEVKFNWYVDGVEVHNAKTKPREEQYNSTYRVVSVLTVLHQDWLNGKEYKCKVSNKALPAPIEKTISKAKGQPREPQVYTLPPSRDELTKNQVSLTCLVKGFYPSDIAVEWESNGQPENNYKTTPPVLDSDGSFFLYSKLTVDKSRWQQGNVFSCSVMHEALHNHYTQKSLSLSPGK

SEQ ID NO: 3 - DNA, 1707 bp, Artificial Sequence
  838 molecule nucleic acid sequence
atggagagcaaggtgctgctggccgtcgccctgtggctctgcgtggagacccgggccgcctctgtgggtttgcctagtgtttctcttgatctgcccaggctcagcatacaaaaagacatacttacaattaaggctaatacaactcttcaaattacttgcaggggacagagggacttggactggctttggcccaataatcagagtggcagtgagcaaagggtggaggtgactgagtgcagcgatggcctcttctgtaagacactcacaattccaaaagtgatcggaaatgacactggagcctacaagtgcttctaccgggaaactgacttggcctcggtcatttatgtctatgttcaagattacagatctccatttattgcttctgttagtgaccaacatggagtcgtgtacattactgagaacaaaaacaaaactgtggtgattccatgtctcgggtccatttcaaatctcaacgtgtcactttgtgcaagatacccagaaaagagatttgttcctgatggtaacagaatttcctgggacagcaagaagggctttactattcccagctacatgatcagctatgctggcatggtcttctgtgaagcaaaaattaatgatgaaagttaccagtctattatgtacatagttgtcgttgtagggtataggatttatgatgtggttctgagtccgtctcatggaattgaactatctgttggagaaaagcttgtcttaaattgtacagcaagaactgaactaaatgtggggattgacttcaactgggaatacccttcttcgaagcatcagcataagaaacttgtaaaccgagacctaaaaacccagtctgggagtgagatgaagaaatttttgagcaccttaactatagatggtgtaacccggagtgaccaaggattgtacacctgtgcagcatccagtgggctgatgaccaagaagaacagcacatttgtcagggtccatgaaaaaccttttgttgcttttggaagtggcgaattcgagcccaaatcttgtgacaaaactcacacatgcccaccgtgcccagcacctgaactcctggggggaccgtcagtcttcctcttccccccaaaacccaaggacaccctcatgatctcccggacccctgaggtcacatgcgtggtggtggacgtgagccacgaagaccctgaggtcaagttcaactggtacgtggacggcgtggaggtgcataatgccaagacaaagccgcgggaggagcagtacaacagcacgtaccgtgtggtcagcgtcctcaccgtcctgcaccaggactggctgaatggcaaggagtacaagtgcaaggtctccaacaaagccctcccagcccccatcgagaaaaccatctccaaagccaaagggcagccccgagaaccacaggtgtacaccctgcccccatcccgggatgagctgaccaagaaccaggtcagcctgacctgcctggtcaaaggcttctatcccagcgacatcgccgtggagtgggagagcaatgggcagccggagaacaactacaagaccacgcctcccgtgctggactccgacggctccttcttcctctacagcaagctcaccgtggacaagagcaggtggcagcaggggaacgtcttctcatgctccgtgatgcatgaggctctgcacaaccactacacgcagaagagcctctccctgtctccgggtaaa

SEQ ID NO: 4 - protein, 569 aa, Artificial Sequence
  838 molecule amino acid sequence
MESKVLLAVALWLCVETRAASVGLPSVSLDLPRLSIQKDILTIKANTTLQITCRGQRDLDWLWPNNQSGSEQRVEVTECSDGLFCKTLTIPKVIGNDTGAYKCFYRETDLASVIYVYVQDYRSPFIASVSDQHGVVYITENKNKTVVIPCLGSISNLNVSLCARYPEKRFVPDGNRISWDSKKGFTIPSYMISYAGMVFCEAKINDESYQSIMYIVVVVGYRIYDVVLSPSHGIELSVGEKLVLNCTARTELNVGIDFNWEYPSSKHQHKKLVNRDLKTQSGSEMKKFLSTLTIDGVTRSDQGLYTCAASSGLMTKKNSTFVRVHEKPFVAFGSGEFEPKSCDKTHTCPPCPAPELLGGPSVFLFPPKPKDTLMISRTPEVTCVVVDVSHEDPEVKFNWYVDGVEVHNAKTKPREEQYNSTYRVVSVLTVLHQDWLNGKEYKCKVSNKALPAPIEKTISKAKGQPREPQVYTLPPSRDELTKNQVSLTCLVKGFYPSDIAVEWESNGQPENNYKTTPPVLDSDGSFFLYSKLTVDKSRWQQGNVFSCSVMHEALHNHYTQKSLSLSPGK

SEQ ID NO: 5 - DNA, 858 bp, Artificial Sequence
  876 molecule nucleic acid sequence
atggacatgcgggtgccagctcagctgctgggactgctgctgctgtggctgcccggcaccagatgcgacatccagctgacccagtccccctccagcctgtccgcctctgtgggcgacagagtgaccatcacctgttccgcctcccaggacatcagcaactacctgaactggtatcagcagaagcccggcaaggcccccaaggtgctgatctacttcaccagcagcctgcactccggcgtgccctcccggttctccggctccggctccggcaccgacttcaccctgaccatctccagcctgcagcccgaggacttcgccacctactactgccagcagtacagcaccgtgccctggaccttcggccagggcaccaaggtggaaatcaagggaggtggaggaagcggtggaggaggtagcggaggcggcggcagcgaggtgcagctggtggaatccggcggaggactggtgcagcctggcggctccctgagactgtcttgcgccgcctccggctacgacttcacccactacggcatgaactgggtccgacaggcccctggcaagggactggaatgggtgggctggatcaacacctacaccggcgagcccacctacgccgccgacttcaagcggcggttcaccttcagcctggacaccagcaagagcaccgcctacctgcagatgaactccctgcgggccgaggacaccgccgtgtactactgcgccaagtacccctactactacggcaccagccactggtacttcgacgtgtggggccagggcaccctggtcaccgtctcctcacaccatcaccaccaccacaccctggtcaccgtctcctcacaccatcaccaccaccac

SEQ ID NO: 6 - protein, 273 aa, Artificial Sequence
  876 molecule amino acid sequence
MDMRVPAQLLGLLLLWLPGTRCDIQLTQSPSSLSASVGDRVTITCSASQDISNYLNWYQQKPGKAPKVLIYFTSSLHSGVPSRFSGSGSGTDFTLTISSLQPEDFATYYCQQYSTVPWTFGQGTKVEIKGGGGSGGGGSGGGGSEVQLVESGGGLVQPGGSLRLSCAASGYDFTHYGMNWVRQAPGKGLEWVGWINTYTGEPTYAADFKRRFTFSLDTSKSTAYLQMNSLRAEDTAVYYCAKYPYYYGTSHWYFDVWGQGTLVTVSSHHHHHH

SEQ ID NO: 7 - DNA, 1371 bp, Artificial Sequence
  873 molecule nucleic acid sequence
atggtcagctactgggacaccggggtcctgctgtgcgcgctgctcagctgtctgcttctcacaggatctagttcaggtagtgatacaggtagacctttcgtagagatgtacagtgaaatccccgaaattatacacatgactgaaggaagggagctcgtcattccctgccgggttacgtcacctaacatcactgttactttaaaaaagtttccacttgacactttgatccctgatggaaaacgcataatctgggacagtagaaagggcttcatcatatcaaatgcaacgtacaaagaaatagggcttctgacctgtgaagcaacagtcaatgggcatttgtataagacaaactatctcacacatcgacaaaccaatacaatcatcgatgtggttctgagtccgtctcatggaattgaactatctgttggagaaaagcttgtcttaaattgtacagcaagaactgaactaaatgtggggattgacttcaactgggaatacccttcttcgaagcatcagcataagaaacttgtaaaccgagacctaaaaacccagtctgggagtgagatgaagaaatttttgagcaccttaactatagatggtgtaacccggagtgaccaaggattgtacacctgtgcagcatccagtgggctgatgaccaagaagaacagcacatttgtcagggtccatgaaaaagacaaaactcacacatgcccaccgtgcccagcacctgaactcctggggggaccgtcagtcttcctcttccccccaaaacccaaggacaccctcatgatctcccggacccctgaggtcacatgcgtggtggtggacgtgagccacgaagaccctgaggtcaagttcaactggtacgtggacggcgtggaggtgcataatgccaagacaaagccgcgggaggagcagtacaacagcacgtaccgtgtggtcagcgtcctcaccgtcctgcaccaggactggctgaatggcaaggagtacaagtgcaaggtctccaacaaagccctcccagcccccatcgagaaaaccatctccaaagccaaagggcagccccgagaaccacaggtgtacaccctgcccccatcccgggatgagctgaccaagaaccaggtcagcctgacctgcctggtcaaaggcttctatcccagcgacatcgccgtggagtgggagagcaatgggcagccggagaacaactacaagaccacgcctcccgtgctggactccgacggctccttcttcctctacagcaagctcaccgtggacaagagcaggtggcagcaggggaacgtcttctcatgctccgtgatgcatgaggctctgcacaaccactacacgcagaagagcctctccctgtctccgggt

SEQ ID NO: 8 - protein, 457 aa, Artificial Sequence
  873 molecule amino acid sequence
MVSYWDTGVLLCALLSCLLLTGSSSGSDTGRPFVEMYSEIPEIIHMTEGRELVIPCRVTSPNITVTLKKFPLDTLIPDGKRIIWDSRKGFIISNATYKEIGLLTCEATVNGHLYKTNYLTHRQTNTIIDVVLSPSHGIELSVGEKLVLNCTARTELNVGIDFNWEYPSSKHQHKKLVNRDLKTQSGSEMKKFLSTLTIDGVTRSDQGLYTCAASSGLMTKKNSTFVRVHEKDKTHTCPPCPAPELLGGPSVFLFPPKPKDTLMISRTPEVTCVVVDVSHEDPEVKFNWYVDGVEVHNAKTKPREEQYNSTYRVVSVLTVLHQDWLNGKEYKCKVSNKALPAPIEKTISKAKGQPREPQVYTLPPSRDELTKNQVSLTCLVKGFYPSDIAVEWESNGQPENNYKTTPPVLDSDGSFFLYSKLTVDKSRWQQGNVFSCSVMHEALHNHYTQKSLSLSPG

SEQ ID NO: 9 - DNA, 1416 bp, Artificial Sequence
  874 molecule nucleic acid sequence
atggactggacctggtctatcctgttcctggtggccgctgcaaccggcacctactccgaggtgcagctggtggaatccggcggaggactggtgcagcctggcggctccctgagactgtcttgcgccgcctccggctacaccttcaccaactacggcatgaactgggtccgacaggcccctggcaagggactggaatgggtgggctggatcaacacctacaccggcgagcccacctacgccgccgacttcaagcggcggttcaccttcagcctggacaccagcaagagcaccgcctacctgcagatgaactccctgcgggccgaggacaccgccgtgtactactgcgccaagtacccccactactacggcagcagccactggtacttcgacgtgtggggccagggcaccctggtcaccgtctcctcagcctccaccaagggcccatcggtcttccccctggcaccctcctccaagagcacctctgggggcacagcggccctgggctgcctggtcaaggactacttccccgaaccggtgacggtgtcgtggaactcaggcgccctgaccagcggcgtgcacaccttcccggctgtcctacagtcctcaggactctactccctcagcagcgtggtgaccgtgccctccagcagcttgggcacccagacctacatctgcaacgtgaatcacaagcccagcaacaccaaggtggacaagaaagttgagcccaaatcttgtgacaaaactcacacatgcccaccgtgcccagcacctgaactcctggggggaccgtcagtcttcctcttccccccaaaacccaaggacaccctcatgatctcccggacccctgaggtcacatgcgtggtggtggacgtgagccacgaagaccctgaggtcaagttcaactggtacgtggacggcgtggaggtgcataatgccaagacaaagccgcgggaggagcagtacaacagcacgtaccgtgtggtcagcgtcctcaccgtcctgcaccaggactggctgaatggcaaggagtacaagtgcaaggtctccaacaaagccctcccagcccccatcgagaaaaccatctccaaagccaaagggcagccccgagaaccacaggtgtacaccctgcccccatcccgggatgagctgaccaagaaccaggtcagcctgacctgcctggtcaaaggcttctatcccagcgacatcgccgtggagtgggagagcaatgggcagccggagaacaactacaagaccacgcctcccgtgctggactccgacggctccttcttcctctacagcaagctcaccgtggacaagagcaggtggcagcaggggaacgtcttctcatgctccgtgatgcatgaggctctgcacaaccactacacgcagaagagcctctccctgtctccgggtaaa

SEQ ID NO: 10 - protein, 472 aa, Artificial Sequence
  874 molecule amino acid sequence
MDWTWSILFLVAAATGTYSEVQLVESGGGLVQPGGSLRLSCAASGYTFTNYGMNWVRQAPGKGLEWVGWINTYTGEPTYAADFKRRFTFSLDTSKSTAYLQMNSLRAEDTAVYYCAKYPHYYGSSHWYFDVWGQGTLVTVSSASTKGPSVFPLAPSSKSTSGGTAALGCLVKDYFPEPVTVSWNSGALTSGVHTFPAVLQSSGLYSLSSVVTVPSSSLGTQTYICNVNHKPSNTKVDKKVEPKSCDKTHTCPPCPAPELLGGPSVFLFPPKPKDTLMISRTPEVTCVVVDVSHEDPEVKFNWYVDGVEVHNAKTKPREEQYNSTYRVVSVLTVLHQDWLNGKEYKCKVSNKALPAPIEKTISKAKGQPREPQVYTLPPSRDELTKNQVSLTCLVKGFYPSDIAVEWESNGQPENNYKTTPPVLDSDGSFFLYSKLTVDKSRWQQGNVFSCSVMHEALHNHYTQKSLSLSPGK

SEQ ID NO: 11 - DNA, 708 bp, Artificial Sequence
  875 molecule nucleic acid sequence
atggacatgcgggtgccagctcagctgctgggactgctgctgctgtggctgcccggcaccagatgcgacatccagatgacccagtccccctccagcctgtccgcctctgtgggcgacagagtgaccatcacctgttccgcctcccaggacatcagcaactacctgaactggtatcagcagaagcccggcaaggcccccaaggtgctgatctacttcaccagcagcctgcactccggcgtgccctcccggttctccggctccggctccggcaccgacttcaccctgaccatctccagcctgcagcccgaggacttcgccacctactactgccagcagtacagcaccgtgccctggaccttcggccagggcaccaaggtggaaatcaagcggaccgtggccgctccctccgtgttcatcttcccaccctccgacgagcagctgaagtccggcaccgcctccgtcgtctgcctgctgaacaacttctacccccgcgaggccaaggtgcagtggaaggtggacaacgccctgcagtccggcaactcccaggaatccgtcaccgagcaggactccaaggacagcacctactccctgtcctccaccctgaccctgtccaaggccgactacgagaagcacaaggtgtacgcctgcgaagtgacccaccagggcctgtccagccccgtgaccaagtccttcaaccggggcgagtgc

SEQ ID NO: 12 - protein, 236 aa, Artificial Sequence
  875 molecule amino acid sequence
MDMRVPAQLLGLLLLWLPGTRCDIQMTQSPSSLSASVGDRVTITCSASQDISNYLNWYQQKPGKAPKVLIYFTSSLHSGVPSRFSGSGSGTDFTLTISSLQPEDFATYYCQQYSTVPWTFGQGTKVEIKRTVAAPSVFIFPPSDEQLKSGTASVVCLLNNFYPREAKVQWKVDNALQSGNSQESVTEQDSKDSTYSLSSTLTLSKADYEKHKVYACEVTHQGLSSPVTKSFNRGEC

SEQ ID NO: 13 - DNA, 750 bp, Artificial Sequence
  915 molecule nucleic acid sequence
atggactggacctggtctatcctgttcctggtggccgctgcaaccggcacctactccgaggtgcagctggtggaatccggcggaggactggtgcagcctggcggctccctgagactgtcttgcgccgcctccggctacgacttcacccactacggcatgaactgggtccgacaggcccctggcaagggactggaatgggtgggctggatcaacacctacaccggcgagcccacctacgccgccgacttcaagcggcggttcaccttcagcctggacaccagcaagagcaccgcctacctgcagatgaactccctgcgggccgaggacaccgccgtgtactactgcgccaagtacccctactactacggcaccagccactggtacttcgacgtgtggggccagggcaccctggtcaccgtctcctcagcctccaccaagggcccatcggtcttccccctggcaccctcctccaagagcacctctgggggcacagcggccctgggctgcctggtcaaggactacttccccgaaccggtgacggtgtcgtggaactcaggcgccctgaccagcggcgtgcacaccttcccggctgtcctacagtcctcaggactctactccctcagcagcgtggtgaccgtgccctccagcagcttgggcacccagacctacatctgcaacgtgaatcacaagcccagcaacaccaaggtggacaagaaagttgagcccaaatcttgtgacaaaactcacctg

SEQ ID NO: 14 - protein, 250 aa, Artificial Sequence
  915 molecule amino acid sequence
MDWTWSILFLVAAATGTYSEVQLVESGGGLVQPGGSLRLSCAASGYDFTHYGMNWVRQAPGKGLEWVGWINTYTGEPTYAADFKRRFTFSLDTSKSTAYLQMNSLRAEDTAVYYCAKYPYYYGTSHWYFDVWGQGTLVTVSSASTKGPSVFPLAPSSKSTSGGTAALGCLVKDYFPEPVTVSWNSGALTSGVHTFPAVLQSSGLYSLSSVVTVPSSSLGTQTYICNVNHKPSNTKVDKKVEPKSCDKTHL

SEQ ID NO: 15 - DNA, 708 bp, Artificial Sequence
  914 molecule nucleic acid sequence
atggacatgcgggtgccagctcagctgctgggactgctgctgctgtggctgcccggcaccagatgcgacatccagctgacccagtccccctccagcctgtccgcctctgtgggcgacagagtgaccatcacctgttccgcctcccaggacatcagcaactacctgaactggtatcagcagaagcccggcaaggcccccaaggtgctgatctacttcaccagcagcctgcactccggcgtgccctcccggttctccggctccggctccggcaccgacttcaccctgaccatctccagcctgcagcccgaggacttcgccacctactactgccagcagtacagcaccgtgccctggaccttcggccagggcaccaaggtggaaatcaagcggaccgtggccgctccctccgtgttcatcttcccaccctccgacgagcagctgaagtccggcaccgcctccgtcgtctgcctgctgaacaacttctacccccgcgaggccaaggtgcagtggaaggtggacaacgccctgcagtccggcaactcccaggaatccgtcaccgagcaggactccaaggacagcacctactccctgtcctccaccctgaccctgtccaaggccgactacgagaagcacaaggtgtacgcctgcgaagtgacccaccagggcctgtccagccccgtgaccaagtccttcaaccggggcgagtgc

SEQ ID NO: 16 - protein, 236 aa, Artificial Sequence
  914 molecule amino acid sequence
MDMRVPAQLLGLLLLWLPGTRCDIQLTQSPSSLSASVGDRVTITCSASQDISNYLNWYQQKPGKAPKVLIYFTSSLHSGVPSRFSGSGSGTDFTLTISSLQPEDFATYYCQQYSTVPWTFGQGTKVEIKRTVAAPSVFIFPPSDEQLKSGTASVVCLLNNFYPREAKVQWKVDNALQSGNSQESVTEQDSKDSTYSLSSTLTLSKADYEKHKVYACEVTHQGLSSPVTKSFNRGEC

SEQ ID NO: 17 - DNA, 1416 bp, Artificial Sequence
  916 molecule nucleic acid sequence
atggactggacctggtctatcctgttcctggtggccgctgcaaccggcacctactccgaggtgcagctggtggaatccggcggaggactggtgcagcctggcggctccctgagactgtcttgcgccgcctccggctacgacttcacccactacggcatgaactgggtccgacaggcccctggcaagggactggaatgggtgggctggatcaacacctacaccggcgagcccacctacgccgccgacttcaagcggcggttcaccttcagcctggacaccagcaagagcaccgcctacctgcagatgaactccctgcgggccgaggacaccgccgtgtactactgcgccaagtacccctactactacggcaccagccactggtacttcgacgtgtggggccagggcaccctggtcaccgtctcctcagcctccaccaagggcccatcggtcttccccctggcaccctcctccaagagcacctctgggggcacagcggccctgggctgcctggtcaaggactacttccccgaaccggtgacggtgtcgtggaactcaggcgccctgaccagcggcgtgcacaccttcccggctgtcctacagtcctcaggactctactccctcagcagcgtggtgaccgtgccctccagcagcttgggcacccagacctacatctgcaacgtgaatcacaagcccagcaacaccaaggtggacaagaaagttgagcccaaatcttgtgacaaaactcacacatgcccaccgtgcccagcacctgaactcctggggggaccgtcagtcttcctcttccccccaaaacccaaggacaccctcatgatctcccggacccctgaggtcacatgcgtggtggtggacgtgagccacgaagaccctgaggtcaagttcaactggtacgtggacggcgtggaggtgcataatgccaagacaaagccgcgggaggagcagtacaacagcacgtaccgtgtggtcagcgtcctcaccgtcctgcaccaggactggctgaatggcaaggagtacaagtgcaaggtctccaacaaagccctcccagcccccatcgagaaaaccatctccaaagccaaagggcagccccgagaaccacaggtgtacaccctgcccccatcccgggatgagctgaccaagaaccaggtcagcctgacctgcctggtcaaaggcttctatcccagcgacatcgccgtggagtgggagagcaatgggcagccggagaacaactacaagaccacgcctcccgtgctggactccgacggctccttcttcctctacagcaagctcaccgtggacaagagcaggtggcagcaggggaacgtcttctcatgctccgtgatgcatgaggctctgcacaaccactacacgcagaagagcctctccctgtctccgggtaaa

SEQ ID NO: 18 - protein, 472 aa, Artificial Sequence
  916 molecule amino acid sequence
MDWTWSILFLVAAATGTYSEVQLVESGGGLVQPGGSLRLSCAASGYDFTHYGMNWVRQAPGKGLEWVGWINTYTGEPTYAADFKRRFTFSLDTSKSTAYLQMNSLRAEDTAVYYCAKYPYYYGTSHWYFDVWGQGTLVTVSSASTKGPSVFPLAPSSKSTSGGTAALGCLVKDYFPEPVTVSWNSGALTSGVHTFPAVLQSSGLYSLSSVVTVPSSSLGTQTYICNVNHKPSNTKVDKKVEPKSCDKTHTCPPCPAPELLGGPSVFLFPPKPKDTLMISRTPEVTCVVVDVSHEDPEVKFNWYVDGVEVHNAKTKPREEQYNSTYRVVSVLTVLHQDWLNGKEYKCKVSNKALPAPIEKTISKAKGQPREPQVYTLPPSRDELTKNQVSLTCLVKGFYPSDIAVEWESNGQPENNYKTTPPVLDSDGSFFLYSKLTVDKSRWQQGNVFSCSVMHEALHNHYTQKSLSLSPGK

SEQ ID NO: 19 - DNA, 801 bp, Artificial Sequence
  913 molecule nucleic acid sequence
atggacatgcgggtgccagctcagctgctgggactgctgctgctgtggctgcccggcaccagatgcgacatccagctgacccagtccccctccagcctgtccgcctctgtgggcgacagagtgaccatcacctgttccgcctcccaggacatcagcaactacctgaactggtatcagcagaagcccggcaaggcccccaaggtgctgatctacttcaccagcagcctgcactccggcgtgccctcccggttctccggctccggctccggcaccgacttcaccctgaccatctccagcctgcagcccgaggacttcgccacctactactgccagcagtacagcaccgtgccctggaccttcggccagggcaccaaggtggaaatcaagggaggtggaggaagcggtggaggaggtagcggaggcggcggcagcgaggtgcagctggtggaatccggcggaggactggtgcagcctggcggctccctgagactgtcttgcgccgcctccggctacgacttcacccactacggcatgaactgggtccgacaggcccctggcaagggactggaatgggtgggctggatcaacacctacaccggcgagcccacctacgccgccgacttcaagcggcggttcaccttcagcctggacaccagcaagagcaccgcctacctgcagatgaactccctgcgggccgaggacaccgccgtgtactactgcgccaagtacccctactactacggcaccagccactggtacttcgacgtgtggggccagggcaccctggtcaccgtctcctca

SEQ ID NO: 20 - protein, 267 aa, Artificial Sequence
  913 molecule amino acid sequence
MDMRVPAQLLGLLLLWLPGTRCDIQLTQSPSSLSASVGDRVTITCSASQDISNYLNWYQQKPGKAPKVLIYFTSSLHSGVPSRFSGSGSGTDFTLTISSLQPEDFATYYCQQYSTVPWTFGQGTKVEIKGGGGSGGGGSGGGGSEVQLVESGGGLVQPGGSLRLSCAASGYDFTHYGMNWVRQAPGKGLEWVGWINTYTGEPTYAADFKRRFTFSLDTSKSTAYLQMNSLRAEDTAVYYCAKYPYYYGTSHWYFDVWGQGTLVTVSS

SEQ ID NO: 21 - DNA, 1377 bp, Artificial Sequence
  917 molecule nucleic acid sequence
atggtcagctactgggacaccggggtcctgctgtgcgcgctgctcagctgtctgcttctcacaggatctagttcaggttcgcgaagtgatacaggtagacctttcgtagagatgtacagtgaaatccccgaaattatacacatgactgaaggaagggagctcgtcattccctgccgggttacgtcacctaacatcactgttactttaaaaaagtttccacttgacactttgatccctgatggaaaacgcataatctgggacagtagaaagggcttcatcatatcaaatgcaacgtacaaagaaatagggcttctgacctgtgaagcaacagtcaatgggcatttgtataagacaaactatctcacacatcgacaaaccaatacaatcatcgatgtggttctgagtccgtctcatggaattgaactatctgttggagaaaagcttgtcttaaattgtacagcaagaactgaactaaatgtggggattgacttcaactgggaatacccttcttcgaagcatcagcataagaaacttgtaaaccgagacctaaaaacccagtctgggagtgagatgaagaaatttttgagcaccttaactatagatggtgtaacccggagtgaccaaggattgtacacctgtgcagcatccagtgggctgatgaccaagaagaacagcacatttgtcagggtccatgaaaaagacaaaactcacacatgcccaccgtgcccagcacctgaactcctggggggaccgtcagtcttcctcttccccccaaaacccaaggacaccctcatgatctcccggacccctgaggtcacatgcgtggtggtggacgtgagccacgaagaccctgaggtcaagttcaactggtacgtggacggcgtggaggtgcataatgccaagacaaagccgcgggaggagcagtacaacagcacgtaccgtgtggtcagcgtcctcaccgtcctgcaccaggactggctgaatggcaaggagtacaagtgcaaggtctccaacaaagccctcccagcccccatcgagaaaaccatctccaaagccaaagggcagccccgagaaccacaggtgtacaccctgcccccatcccgggatgagctgaccaagaaccaggtcagcctgacctgcctggtcaaaggcttctatcccagcgacatcgccgtggagtgggagagcaatgggcagccggagaacaactacaagaccacgcctcccgtgctggactccgacggctccttcttcctctacagcaagctcaccgtggacaagagcaggtggcagcaggggaacgtcttctcatgctccgtgatgcatgaggctctgcacaaccactacacgcagaagagcctctccctgtctccgggt

SEQ ID NO: 22 - protein, 459 aa, Artificial Sequence
  917 molecule amino acid sequence
MVSYWDTGVLLCALLSCLLLTGSSSGSRSDTGRPFVEMYSEIPEIIHMTEGRELVIPCRVTSPNITVTLKKFPLDTLIPDGKRIIWDSRKGFIISNATYKEIGLLTCEATVNGHLYKTNYLTHRQTNTIIDVVLSPSHGIELSVGEKLVLNCTARTELNVGIDFNWEYPSSKHQHKKLVNRDLKTQSGSEMKKFLSTLTIDGVTRSDQGLYTCAASSGLMTKKNSTFVRVHEKDKTHTCPPCPAPELLGGPSVFLFPPKPKDTLMISRTPEVTCVVVDVSHEDPEVKFNWYVDGVEVHNAKTKPREEQYNSTYRVVSVLTVLHQDWLNGKEYKCKVSNKALPAPIEKTISKAKGQPREPQVYTLPPSRDELTKNQVSLTCLVKGFYPSDIAVEWESNGQPENNYKTTPPVLDSDGSFFLYSKLTVDKSRWQQGNVFSCSVMHEALHNHYTQKSLSLSPG

SEQ ID NO: 23 - DNA, 2265 bp, Artificial Sequence
  964 molecule nucleic acid sequence
atgcggcttccgggtgcgatgccagctctggccctcaaaggcgagctgctgttgctgtctctcctgttacttctggaaccacagatctctcagggcctggtcgtcacacccccggggccagagcttgtcctcaatgtctccagcaccttcgttctgacctgctcgggttcagctccggtggtgtgggaacggatgtcccaggagcccccacaggaaatggccaaggcccaggatggcaccttctccagcgtgctcacactgaccaacctcactgggctagacacgggagaatacttttgcacccacaatgactcccgtggactggagaccgatgagcggaaacggctctacatctttgtgccagatcccaccgtgggcttcctccctaatgatgccgaggaactattcatctttctcacggaaataactgagatcaccattccatgccgagtaacagacccacagctggtggtgacactgcacgagaagaaaggggacgttgcactgcctgtcccctatgatcaccaacgtggcttttctggtatctttgaggacagaagctacatctgcaaaaccaccattggggacagggaggtggattctgatgcctactatgtctacagactccaggtgtcatccatcaacgtctctgtgaacgcagtgcagactgtggtccgccagggtgagaacatcaccctcatgtgcattgtgatcgggaatgaggtggtcaacttcgagtggacatacccccgcaaagaaagtgggcggctggtggagccggtgactgacttcctcttggatatgccttaccacatccgctccatcctgcacatccccagtgccgagttagaagactcggggacctacacctgcaatgtgacggagagtgtgaatgaccatcaggatgaaaaggccatcaacatcaccgtggttgagagcggctacgtgcggctcctgggagaggtgggcacactacaatttgctgagctgcatcggagccggacactgcaggtagtgttcgaggcctacccaccgcccactgtcctgtggttcaaagacaaccgcaccctgggcgactccagcgctggcgaaatcgccctgtccacgcgcaacgtgtcggagacccggtatgtgtcagagctgacactggttcgcgtgaaggtggcagaggctggccactacaccatgcgggccttccatgaggatgctgaggtccagctctccttccagctacagatcaatgtccctgtccgagtgctggagctaagtgagagccaccctgacagtggggaacagacagtccgctgtcgtggccggggcatgccccagccgaacatcatctggtctgcctgcagagacctcaaaaggtgtccacgtgagctgccgcccacgctgctggggaacagttccgaagaggagagccagctggagactaacgtgacgtactgggaggaggagcaggagtttgaggtggtgagcacactgcgtctgcagcacgtggatcggccactgtcggtgcgctgcacgctgcgcaacgctgtgggccaggacacgcaggaggtcatcgtggtgccacactccttgcccttcaagcccccatgcccatcatgcccagcacctgagttcctggggggaccatcagtcttcctgttccccccaaaacccaaggacactctcatgatctcccggacccctgaggtcacgtgcgtggtggtggacgtgagccaggaagaccccgaggtccagttcaactggtacgtggatggcgtggaggtgcataatgccaagacaaagccgcgggaggagcagttcaacagcacgtaccgtgtggtcagcgtcctcaccgtcctgcaccaggactggctgaacggcaaggagtacaagtgcaaggtctccaacaaaggcctcccgtcctccatcgagaaaaccatctccaaagccaaagggcagccccgagagccacaggtgtacaccctgcccccatcccaggaggagatgaccaagaaccaggtcagcctgacctgcctggtcaaaggcttctaccccagcgacatcgccgtggagtgggagagcaatgggcagccggagaacaactacaagaccacgcctcccgtgctggactccgacggctccttcttcctctacagcaggctaaccgtggacaagagcaggtggcaggaggggaatgtcttctcatgctccgtgatgcatgaggctctgcacaaccactacacacagaagagcctctccctgtctctgggtaaa

SEQ ID NO: 24 - protein, 755 aa, Artificial Sequence
  964 molecule amino acid sequence
MRLPGAMPALALKGELLLLSLLLLLEPQISQGLVVTPPGPELVLNVSSTFVLTCSGSAPVVWERMSQEPPQEMAKAQDGTFSSVLTLTNLTGLDTGEYFCTHNDSRGLETDERKRLYIFVPDPTVGFLPNDAEELFIFLTEITEITIPCRVTDPQLVVTLHEKKGDVALPVPYDHQRGFSGIFEDRSYICKTTIGDREVDSDAYYVYRLQVSSINVSVNAVQTVVRQGENITLMCIVIGNEVVNFEWTYPRKESGRLVEPVTDFLLDMPYHIRSILHIPSAELEDSGTYTCNVTESVNDHQDEKAINITVVESGYVRLLGEVGTLQFAELHRSRTLQVVFEAYPPPTVLWFKDNRTLGDSSAGEIALSTRNVSETRYVSELTLVRVKVAEAGHYTMRAFHEDAEVQLSFQLQINVPVRVLELSESHPDSGEQTVRCRGRGMPQPNIIWSACRDLKRCPRELPPTLLGNSSEEESQLETNVTYWEEEQEFEVVSTLRLQHVDRPLSVRCTLRNAVGQDTQEVIVVPHSLPFKPPCPSCPAPEFLGGPSVFLFPPKPKDTLMISRTPEVTCVVVDVSQEDPEVQFNWYVDGVEVHNAKTKPREEQFNSTYRVVSVLTVLHQDWLNGKEYKCKVSNKGLPSSIEKTISKAKGQPREPQVYTLPPSQEEMTKNQVSLTCLVKGFYPSDIAVEWESNGQPENNYKTTPPVLDSDGSFFLYSRLTVDKSRWQEGNVFSCSVMHEALHNHYTQKSLSLSLGK

SEQ ID NO: 25 - DNA, 2295 bp, Artificial Sequence
  963 molecule nucleic acid sequence
atgcggcttccgggtgcgatgccagctctggccctcaaaggcgagctgctgttgctgtctctcctgttacttctggaaccacagatctctcagggcctggtcgtcacacccccggggccagagcttgtcctcaatgtctccagcaccttcgttctgacctgctcgggttcagctccggtggtgtgggaacggatgtcccaggagcccccacaggaaatggccaaggcccaggatggcaccttctccagcgtgctcacactgaccaacctcactgggctagacacgggagaatacttttgcacccacaatgactcccgtggactggagaccgatgagcggaaacggctctacatctttgtgccagatcccaccgtgggcttcctccctaatgatgccgaggaactattcatctttctcacggaaataactgagatcaccattccatgccgagtaacagacccacagctggtggtgacactgcacgagaagaaaggggacgttgcactgcctgtcccctatgatcaccaacgtggcttttctggtatctttgaggacagaagctacatctgcaaaaccaccattggggacagggaggtggattctgatgcctactatgtctacagactccaggtgtcatccatcaacgtctctgtgaacgcagtgcagactgtggtccgccagggtgagaacatcaccctcatgtgcattgtgatcgggaatgaggtggtcaacttcgagtggacatacccccgcaaagaaagtgggcggctggtggagccggtgactgacttcctcttggatatgccttaccacatccgctccatcctgcacatccccagtgccgagttagaagactcggggacctacacctgcaatgtgacggagagtgtgaatgaccatcaggatgaaaaggccatcaacatcaccgtggttgagagcggctacgtgcggctcctgggagaggtgggcacactacaatttgctgagctgcatcggagccggacactgcaggtagtgttcgaggcctacccaccgcccactgtcctgtggttcaaagacaaccgcaccctgggcgactccagcgctggcgaaatcgccctgtccacgcgcaacgtgtcggagacccggtatgtgtcagagctgacactggttcgcgtgaaggtggcagaggctggccactacaccatgcgggccttccatgaggatgctgaggtccagctctccttccagctacagatcaatgtccctgtccgagtgctggagctaagtgagagccaccctgacagtggggaacagacagtccgctgtcgtggccggggcatgccccagccgaacatcatctggtctgcctgcagagacctcaaaaggtgtccacgtgagctgccgcccacgctgctggggaacagttccgaagaggagagccagctggagactaacgtgacgtactgggaggaggagcaggagtttgaggtggtgagcacactgcgtctgcagcacgtggatcggccactgtcggtgcgctgcacgctgcgcaacgctgtgggccaggacacgcaggaggtcatcgtggtgccacactccttgcccttcaaggaccccgagcccaaatcttgtgacaaaactcacacatgcccaccgtgcccagcacctgaactcctggggggaccgtcagtcttcctcttccccccaaaacccaaggacaccctcatgatctcccggacccctgaggtcacatgcgtggtggtggacgtgagccacgaagaccctgaggtcaagttcaactggtacgtggacggcgtggaggtgcataatgccaagacaaagccgcgggaggagcagtacaacagcacgtaccgtgtggtcagcgtcctcaccgtcctgcaccaggactggctgaatggcaaggagtacaagtgcaaggtctccaacaaagccctcccagcccccatcgagaaaaccatctccaaagccaaagggcagccccgagaaccacaggtgtacaccctgcccccatcccgggatgagctgaccaagaaccaggtcagcctgacctgcctggtcaaaggcttctatcccagcgacatcgccgtggagtgggagagcaatgggcagccggagaacaactacaagaccacgcctcccgtgctggactccgacggctccttcttcctctacagcaagctcaccgtggacaagagcaggtggcagcaggggaacgtcttctcatgctccgtgatgcatgaggctctgcacaaccactacacgcagaagagcctctccctgtctccgggtaaa

SEQ ID NO: 26 - protein, 765 aa, Artificial Sequence
  963 molecule amino acid sequence
MRLPGAMPALALKGELLLLSLLLLLEPQISQGLVVTPPGPELVLNVSSTFVLTCSGSAPVVWERMSQEPPQEMAKAQDGTFSSVLTLTNLTGLDTGEYFCTHNDSRGLETDERKRLYIFVPDPTVGFLPNDAEELFIFLTEITEITIPCRVTDPQLVVTLHEKKGDVALPVPYDHQRGFSGIFEDRSYICKTTIGDREVDSDAYYVYRLQVSSINVSVNAVQTVVRQGENITLMCIVIGNEVVNFEWTYPRKESGRLVEPVTDFLLDMPYHIRSILHIPSAELEDSGTYTCNVTESVNDHQDEKAINITVVESGYVRLLGEVGTLQFAELHRSRTLQVVFEAYPPPTVLWFKDNRTLGDSSAGEIALSTRNVSETRYVSELTLVRVKVAEAGHYTMRAFHEDAEVQLSFQLQINVPVRVLELSESHPDSGEQTVRCRGRGMPQPNIIWSACRDLKRCPRELPPTLLGNSSEEESQLETNVTYWEEEQEFEVVSTLRLQHVDRPLSVRCTLRNAVGQDTQEVIVVPHSLPFKDPEPKSCDKTHTCPPCPAPELLGGPSVFLFPPKPKDTLMISRTPEVTCVVVDVSHEDPEVKFNWYVDGVEVHNAKTKPREEQYNSTYRVVSVLTVLHQDWLNGKEYKCKVSNKALPAPIEKTISKAKGQPREPQVYTLPPSRDELTKNQVSLTCLVKGFYPSDIAVEWESNGQPENNYKTTPPVLDSDGSFFLYSKLTVDKSRWQQGNVFSCSVMHEALHNHYTQKSLSLSPGK

SEQ ID NO: 27 - DNA, 1656 bp, Artificial Sequence
  974 molecule nucleic acid sequence
atgcggcttccgggtgcgatgccagctctggccctcaaaggcgagctgctgttgctgtctctcctgttacttctggaaccacagatctctcagggcctggtcgtcacacccccggggccagagcttgtcctcaatgtctccagcaccttcgttctgacctgctcgggttcagctccggtggtgtgggaacggatgtcccaggagcccccacaggaaatggccaaggcccaggatggcaccttctccagcgtgctcacactgaccaacctcactgggctagacacgggagaatacttttgcacccacaatgactcccgtggactggagaccgatgagcggaaacggctctacatctttgtgccagatcccaccgtgggcttcctccctaatgatgccgaggaactattcatctttctcacggaaataactgagatcaccattccatgccgagtaacagacccacagctggtggtgacactgcacgagaagaaaggggacgttgcactgcctgtcccctatgatcaccaacgtggcttttctggtatctttgaggacagaagctacatctgcaaaaccaccattggggacagggaggtggattctgatgcctactatgtctacagactccaggtgtcatccatcaacgtctctgtgaacgcagtgcagactgtggtccgccagggtgagaacatcaccctcatgtgcattgtgatcgggaatgaggtggtcaacttcgagtggacatacccccgcaaagaaagtgggcggctggtggagccggtgactgacttcctcttggatatgccttaccacatccgctccatcctgcacatccccagtgccgagttagaagactcggggacctacacctgcaatgtgacggagagtgtgaatgaccatcaggatgaaaaggccatcaacatcaccgtggttgagagcggctacgtgcggctcctgggagagcccaaatcttgtgacaaaactcacacatgcccaccgtgcccagcacctgaactcctggggggaccgtcagtcttcctcttccccccaaaacccaaggacaccctcatgatctcccggacccctgaggtcacatgcgtggtggtggacgtgagccacgaagaccctgaggtcaagttcaactggtacgtggacggcgtggaggtgcataatgccaagacaaagccgcgggaggagcagtacaacagcacgtaccgtgtggtcagcgtcctcaccgtcctgcaccaggactggctgaatggcaaggagtacaagtgcaaggtctccaacaaagccctcccagcccccatcgagaaaaccatctccaaagccaaagggcagccccgagaaccacaggtgtacaccctgcccccatcccgggatgagctgaccaagaaccaggtcagcctgacctgcctggtcaaaggcttctatcccagcgacatcgccgtggagtgggagagcaatgggcagccggagaacaactacaagaccacgcctcccgtgctggactccgacggctccttcttcctctacagcaagctcaccgtggacaagagcaggtggcagcaggggaacgtcttctcatgctccgtgatgcatgaggctctgcacaaccactacacgcagaagagcctctccctgtctccgggtaaa

SEQ ID NO: 28 - protein, 552 aa, Artificial Sequence
  974 molecule amino acid sequence
MRLPGAMPALALKGELLLLSLLLLLEPQISQGLVVTPPGPELVLNVSSTFVLTCSGSAPVVWERMSQEPPQEMAKAQDGTFSSVLTLTNLTGLDTGEYFCTHNDSRGLETDERKRLYIFVPDPTVGFLPNDAEELFIFLTEITEITIPCRVTDPQLVVTLHEKKGDVALPVPYDHQRGFSGIFEDRSYICKTTIGDREVDSDAYYVYRLQVSSINVSVNAVQTVVRQGENITLMCIVIGNEVVNFEWTYPRKESGRLVEPVTDFLLDMPYHIRSILHIPSAELEDSGTYTCNVTESVNDHQDEKAINITVVESGYVRLLGEPKSCDKTHTCPPCPAPELLGGPSVFLFPPKPKDTLMISRTPEVTCVVVDVSHEDPEVKFNWYVDGVEVHNAKTKPREEQYNSTYRVVSVLTVLHQDWLNGKEYKCKVSNKALPAPIEKTISKAKGQPREPQVYTLPPSRDELTKNQVSLTCLVKGFYPSDIAVEWESNGQPENNYKTTPPVLDSDGSFFLYSKLTVDKSRWQQGNVFSCSVMHEALHNHYTQKSLSLSPGK

SEQ ID NO: 29 - DNA, 1593 bp, Artificial Sequence
  978 molecule nucleic acid sequence
atgcggcttccgggtgcgatgccagctctggccctcaaaggcgagctgctgttgctgtctctcctgttacttctggaaccacagatctctcagggcctggtcgtcacacccccggggccagagcttgtcctcaatgtctccagcaccttcgttctgacctgctcgggttcagctccggtggtgtgggaacggatgtcccaggagcccccacaggaaatggccaaggcccaggatggcaccttctccagcgtgctcacactgaccaacctcactgggctagacacgggagaatacttttgcacccacaatgactcccgtggactggagaccgatgagcggaaacggctctacatctttgtgccagatcccaccgtgggcttcctccctaatgatgccgaggaactattcatctttctcacggaaataactgagatcaccattccatgccgagtaacagacccacagctggtggtgacactgcacgagaagaaaggggacgttgcactgcctgtcccctatgatcaccaacgtggcttttctggtatctttgaggacagaagctacatctgcaaaaccaccattggggacagggaggtggattctgatgcctactatgtctacagactccaggtgtcatccatcaacgtctctgtgaacgcagtgcagactgtggtccgccagggtgagaacatcaccctcatgtgcattgtgatcgggaatgaggtggtcaacttcgagtggacatacccccgcaaagaaagtgggcggctggtggagccggtgactgacttcctcttggatatgccttaccacatccgctccatcctgcacatccccagtgccgagttagaagactcggggacctacacctgcaatgtgacggagagtgtgaatgaccatcaggatgaaaaggccatcaacatcaccgtggttgagagcggctacgtgcggctcctgggagaggtgggcacactacaatttgctgagctgcatcggagccggacactgcaggtagtgttcgaggcctacccaccgcccactgtcctgtggttcaaagacaaccgcaccctgggcgactccagcgctggcgaaatcgccctgtccacgcgcaacgtgtcggagacccggtatgtgtcagagctgacactggttcgcgtgaaggtggcagaggctggccactacaccatgcgggccttccatgaggatgctgaggtccagctctccttccagctacagatcaatgtccctgtccgagtgctggagctaagtgagagccaccctgacagtggggaacagacagtccgctgtcgtggccggggcatgccccagccgaacatcatctggtctgcctgcagagacctcaaaaggtgtccacgtgagctgccgcccacgctgctggggaacagttccgaagaggagagccagctggagactaacgtgacgtactgggaggaggagcaggagtttgaggtggtgagcacactgcgtctgcagcacgtggatcggccactgtcggtgcgctgcacgctgcgcaacgctgtgggccaggacacgcaggaggtcatcgtggtgccacactccttgcccttcaag

SEQ ID NO: 30 - protein, 531 aa, Artificial Sequence
  978 molecule amino acid sequence
MRLPGAMPALALKGELLLLSLLLLLEPQISQGLVVTPPGPELVLNVSSTFVLTCSGSAPVVWERMSQEPPQEMAKAQDGTFSSVLTLTNLTGLDTGEYFCTHNDSRGLETDERKRLYIFVPDPTVGFLPNDAEELFIFLTEITEITIPCRVTDPQLVVTLHEKKGDVALPVPYDHQRGFSGIFEDRSYICKTTIGDREVDSDAYYVYRLQVSSINVSVNAVQTVVRQGENITLMCIVIGNEVVNFEWTYPRKESGRLVEPVTDFLLDMPYHIRSILHIPSAELEDSGTYTCNVTESVNDHQDEKAINITVVESGYVRLLGEVGTLQFAELHRSRTLQVVFEAYPPPTVLWFKDNRTLGDSSAGEIALSTRNVSETRYVSELTLVRVKVAEAGHYTMRAFHEDAEVQLSFQLQINVPVRVLELSESHPDSGEQTVRCRGRGMPQPNIIWSACRDLKRCPRELPPTLLGNSSEEESQLETNVTYWEEEQEFEVVSTLRLQHVDRPLSVRCTLRNAVGQDTQEVIVVPHSLPFK

SEQ ID NO: 31 - DNA, 1737 bp, Artificial Sequence
  977 molecule nucleic acid sequence
atggggcagtgcaggaaaagtggcactatgaaccctgcagccctagacaattgtactaaccttcttctctttcctctcctgacaggttggtgtacagtagcttccaagtactccaccatgcggcttccgggtgcgatgccagctctggccctcaaaggcgagctgctgttgctgtctctcctgttacttctggaaccacagatctctcagggcctggtcgtcacacccccggggccagagcttgtcctcaatgtctccagcaccttcgttctgacctgctcgggttcagctccggtggtgtgggaacggatgtcccaggagcccccacaggaaatggccaaggcccaggatggcaccttctccagcgtgctcacactgaccaacctcactgggctagacacgggagaatacttttgcacccacaatgactcccgtggactggagaccgatgagcggaaacggctctacatctttgtgccagatcccaccgtgggcttcctccctaatgatgccgaggaactattcatctttctcacggaaataactgagatcaccattccatgccgagtaacagacccacagctggtggtgacactgcacgagaagaaaggggacgttgcactgcctgtcccctatgatcaccaacgtggcttttctggtatctttgaggacagaagctacatctgcaaaaccaccattggggacagggaggtggattctgatgcctactatgtctacagactccaggtgtcatccatcaacgtctctgtgaacgcagtgcagactgtggtccgccagggtgagaacatcaccctcatgtgcattgtgatcgggaatgaggtggtcaacttcgagtggacatacccccgcaaagaaagtgggcggctggtggagccggtgactgacttcctcttggatatgccttaccacatccgctccatcctgcacatccccagtgccgagttagaagactcggggacctacacctgcaatgtgacggagagtgtgaatgaccatcaggatgaaaaggccatcaacatcaccgtggttgagagcggctacgtgcggctcctgggagaggtgggcacactacaatttgctgagctgcatcggagccggacactgcaggtagtgttcgaggcctacccaccgcccactgtcctgtggttcaaagacaaccgcaccctgggcgactccagcgctggcgaaatcgccctgtccacgcgcaacgtgtcggagacccggtatgtgtcagagctgacactggttcgcgtgaaggtggcagaggctggccactacaccatgcgggccttccatgaggatgctgaggtccagctctccttccagctacagatcaatgtccctgtccgagtgctggagctaagtgagagccaccctgacagtggggaacagacagtccgctgtcgtggccggggcatgccccagccgaacatcatctggtctgcctgcagagacctcaaaaggtgtccacgtgagctgccgcccacgctgctggggaacagttccgaagaggagagccagctggagactaacgtgacgtactgggaggaggagcaggagtttgaggtggtgagcacactgcgtctgcagcacgtggatcggccactgtcggtgcgctgcacgctgcgcaacgctgtgggccaggacacgcaggaggtcatcgtggtgccacactctttgcccttcaagcggggcagccaccaccaccaccaccac

SEQ ID NO: 32 - protein, 579 aa, Artificial Sequence
  977 molecule amino acid sequence
MGQCRKSGTMNPAALDNCTNLLLFPLLTGWCTVASKYSTMRLPGAMPALALKGELLLLSLLLLLEPQISQGLVVTPPGPELVLNVSSTFVLTCSGSAPVVWERMSQEPPQEMAKAQDGTFSSVLTLTNLTGLDTGEYFCTHNDSRGLETDERKRLYIFVPDPTVGFLPNDAEELFIFLTEITEITIPCRVTDPQLVVTLHEKKGDVALPVPYDHQRGFSGIFEDRSYICKTTIGDREVDSDAYYVYRLQVSSINVSVNAVQTVVRQGENITLMCIVIGNEVVNFEWTYPRKESGRLVEPVTDFLLDMPYHIRSILHIPSAELEDSGTYTCNVTESVNDHQDEKAINITVVESGYVRLLGEVGTLQFAELHRSRTLQVVFEAYPPPTVLWFKDNRTLGDSSAGEIALSTRNVSETRYVSELTLVRVKVAEAGHYTMRAFHEDAEVQLSFQLQINVPVRVLELSESHPDSGEQTVRCRGRGMPQPNIIWSACRDLKRCPRELPPTLLGNSSEEESQLETNVTYWEEEQEFEVVSTLRLQHVDRPLSVRCTLRNAVGQDTQEVIVVPHSLPFKRGSHHHHHH